European Patent Application EP 4 311 858 A1, published January 31, 2024. Title: Intein-based Controllers. Applicant: ETH Zürich. The sequence listing filed with the application follows.

SEQUENCE LISTING (11 sequences)

SEQ ID NO: 1 - protein, 229 aa, synthetic construct
  SOURCE 1..229
MPKKKRKVGSGEFDALDDFDLDMLGSDALDDFDLDMLGSDALDDFDLDMLGSDALDDFDLDMLGSGGGGSGGGGSGGGGSATMMLKKILKIEELDERELIDIEVSGNHLFYANDILTHNSNRGGGGSGGGGSGGGGSGTARPGERPFQCRICMRNFSRQDRLDRHTRTHTGEKPFQCRICMRNFSQKEHLAGHLRTHTGEKPFQCRICMRNFSRRDNLNRHLKTHLRGS

SEQ ID NO: 2 - protein, 239 aa, synthetic construct
  SOURCE 1..239
MPKKKRKVGSGEFDALDDFDLDMLGSDALDDFDLDMLGSDALDDFDLDMLGSDALDDFDLDMLGSGGGGSGGGGSGGGGSATMGSMEAKTYIGKLKSRKIVSNEDTYDIQTSTHNFFANDILVHNSEIGSNRGGGGSGGGGSGGGGSGTARPGERPFQCRICMRNFSRQDRLDRHTRTHTGEKPFQCRICMRNFSQKEHLAGHLRTHTGEKPFQCRICMRNFSRRDNLNRHLKTHLRGS

SEQ ID NO: 3 - protein, 726 aa, synthetic construct
  SOURCE 1..726
MKLLSSIEQACDICRLKKLKCSKEKPKCAKCLKNNWECRYSPKTKRSPLTRAHLTEVESRLERLEGSMLKKILKIEELDERELIDIEVSGNHLFYANDILTHNSGSGSQLFLLIFPREDLDMILKMDSLQDIKALLTGLFVQDNVNKDAVTDRLASVETDMPLTLRQHRISATSSSEESSNKGQRQLTVSGSSEASGSGRADALDDFDLDMLGSDALDDFDLDMLGSDALDDFDLDMLGSDALDDFDLDMLINSRSSGSPKKKRKVGSQYLPDTDDRHRIEEKRKRTYETFKSIMKKSPFSGPTDPRPPPRRIAVPSRSSASVPKPAPQPYPFTSSLSTINYDEFPTMVFPSGQISQASALAPAPPQVLPQAPAPAPAPAMVSALAQAPAPVPVLAPGPPQAVAPPAPKPTQAGEGTLSEALLQLQFDDEDLGALLGNSTDPAVFTDLASVDNSEFQQLLNQGIPVAPHTTEPMLMEYPEAITRLVTGAQRPPDPAPAPLGAPGLPNGLLSGDEDFSSIADMDFSALLGSGSGSRDSREGMFLPKPEAGSAISDVFEGREVCQPKRIRPFHPPGSPWANRPLPASLAPTPTGPVHEPVGSLTPAPVPQPLDPAPAVTPEASHLLEDPDEETSQAVKALREMADTVIPQKEEAAICGQMDLSHPPPRGHLDELTTTLESMTEDLNLDSPLTPELNEILDTFLNDECLLHAMHISTGLSIFDTSLFRS

SEQ ID NO: 4 - protein, 309 aa, synthetic construct
  SOURCE 1..309
MSRLDKSKVINSALELLNEVGIEGLTTRKLAQKLGVEQPTLYWHVKNKRALLDALAIEMLDRHHTHFCPLEGESWQDFLRNKAKSFRCALLSHRDGAKVHLGTRPTEKQYETLENQLAFLCQQGFSLENALYALSAVGHFTLGCVLEDQEHQVAKEERETPTTDSMPPLLRQAIELFDHQGAEPAFLFGLELIICGLEKQLKCESGDSGGGGSMLKKILKIEELDERELIDIEVSGNHLFYANDILTHNSGSGSGRADALDDFDLDMLGSDALDDFDLDMLGSDALDDFDLDMLGSDALDDFDLDMLIN

SEQ ID NO: 5 - protein, 829 aa, synthetic construct
  SOURCE 1..829
MSRLDKSKVINSALELLNEVGIEGLTTRKLAQKLGVEQPTLYWHVKNKRALLDALAIEMLDRHHTHFCPLEGESWQDFLRNNAKSFRCALLSHRDGAKVHLGTRPTEKQYETLENQLAFLCQQGFSLENALYALSAVGHFTLGCVLEDQEHQVAKEERETPTTDSMPPLLRQAIELFDHQGAEPGSMLKKILKIEELDERELIDIEVSGNHLFYANDILTHNSGSGSAFLFGLELIICGLEKQLKCESGSPADALDDFDLDMLPADALDDFDLDMLPADALDDFDLDMLPGQPGSSEASGSGRADALDDFDLDMLGSDALDDFDLDMLGSDALDDFDLDMLGSDALDDFDLDMLINSRSSGSPKKKRKVGSQYLPDTDDRHRIEEKRKRTYETFKSIMKKSPFSGPTDPRPPPRRIAVPSRSSASVPKPAPQPYPFTSSLSTINYDEFPTMVFPSGQISQASALAPAPPQVLPQAPAPAPAPAMVSALAQAPAPVPVLAPGPPQAVAPPAPKPTQAGEGTLSEALLQLQFDDEDLGALLGNSTDPAVFTDLASVDNSEFQQLLNQGIPVAPHTTEPMLMEYPEAITRLVTGAQRPPDPAPAPLGAPGLPNGLLSGDEDFSSIADMDFSALLGSGSGSRDSREGMFLPKPEAGSAISDVFEGREVCQPKRIRPFHPPGSPWANRPLPASLAPTPTGPVHEPVGSLTPAPVPQPLDPAPAVTPEASHLLEDPDEETSQAVKALREMADTVIPQKEEAAICGQMDLSHPPPRGHLDELTTTLESMTEDLNLDSPLTPELNEILDTFLNDECLLHAMHISTGLSIFDTSLFRS

SEQ ID NO: 6 - protein, 285 aa, synthetic construct
  SOURCE 1..285
MSRLDKSKVINSALELLNEVGIEGLTTRKLAQKLGVEQPTLYWHVKNKRALLDALAIEMLDRHHTHFCPLEGESWQDFLRNNAKSFRCALLSHRDGAKVHLGTRPTEKQYETLENQLAFLCQQGFSLENALYALSAVGHFTLGCVLEDQEHQVAKEERETPTTDSMPPLLRQAIELFDHQGAEPAFLFGLELIICGLEKQLKCESGSGGGGSGGGGTGGGGTGTGYNEVLNVFPKSKKKSYKITLEDGKEIICSEEHLFPTQTGEMNISGGLKEGMCLYVKEGST

SEQ ID NO: 7 - protein, 579 aa, synthetic construct
  SOURCE 1..579
MMLKKILKIEELDERELIDIEVSGNHLFYANDILTHNSGSGSSEASGSGRADALDDFDLDMLGSDALDDFDLDMLGSDALDDFDLDMLGSDALDDFDLDMLINSRSSGSPKKKRKVGSQYLPDTDDRHRIEEKRKRTYETFKSIMKKSPFSGPTDPRPPPRRIAVPSRSSASVPKPAPQPYPFTSSLSTINYDEFPTMVFPSGQISQASALAPAPPQVLPQAPAPAPAPAMVSALAQAPAPVPVLAPGPPQAVAPPAPKPTQAGEGTLSEALLQLQFDDEDLGALLGNSTDPAVFTDLASVDNSEFQQLLNQGIPVAPHTTEPMLMEYPEAITRLVTGAQRPPDPAPAPLGAPGLPNGLLSGDEDFSSIADMDFSALLGSGSGSRDSREGMFLPKPEAGSAISDVFEGREVCQPKRIRPFHPPGSPWANRPLPASLAPTPTGPVHEPVGSLTPAPVPQPLDPAPAVTPEASHLLEDPDEETSQAVKALREMADTVIPQKEEAAICGQMDLSHPPPRGHLDELTTTLESMTEDLNLDSPLTPELNEILDTFLNDECLLHAMHISTGLSIFDTSLFRSTSK

SEQ ID NO: 8 - protein, 410 aa, synthetic construct
  SOURCE 1..410
MGGGGSGGGGTGGGGTGTRSGYCLDLKTQVQTPQGMKEISNIQVGDLVLSNTGYNEVLNVFPKSKKKSYKITLEDGKEIICSEEHLFPTQTGEMNISGGLKEGMCLYVKEGSGSGATNFSLLKQAGDVEENPGPGSGEGRGSLLTCGDVEENPGPIDGGSGGSATMVSKGEELFTGVVPILVELDGDVNGHKFSVSGEGEGDATYGKLTLKLICTTGKLPVPWPTLVTTLGYGLQCFARYPDHMKQHDFFKSAMPEGYVQERTIFFKDDGNYKTRAEVKFDGDTLVNRIELKGIDFKEDGNILGHKLEYNYNSHNVYITADKQKNGIKANFKIRHNIEDGGVQLADHYQQNTPIGDGPVLLPDNHYLSYQSKLSKDPNEKRDHMVLLEFVTAAGITLGMDELYKGSGSGS

SEQ ID NO: 9 - protein, 340 aa, synthetic construct
  SOURCE 1..340
MMLKKILKIEELDERELIDIEVSGNHLFYANDILTHNSGSGSGSGATNFSLLKQAGDVEENPGPGSGEGRGSLLTCGDVEENPGPIDGGSGGSATMVSKGEELFTGVVPILVELDGDVNGHKFSVSGEGEGDATYGKLTLKLICTTGKLPVPWPTLVTTLGYGLQCFARYPDHMKQHDFFKSAMPEGYVQERTIFFKDDGNYKTRAEVKFDGDTLVNRIELKGIDFKEDGNILGHKLEYNYNSHNVYITADKQKNGIKANFKIRHNIEDGGVQLADHYQQNTPIGDGPVLLPDNHYLSYQSKLSKDPNEKRDHMVLLEFVTAAGITLGMDELYKGSGSGS

SEQ ID NO: 10 - protein, 409 aa, synthetic construct
  SOURCE 1..409
MNPCCLVGSSEIITRNYGKTTIKEVVEIFDNDKNIQVLAFNTHTDNIEWAPIKAAQLTRPNAELVELEIDTLHGVKTIRCTPDHPVYTKNRGYVRADELTDDDELVVAIGSGSGATNFSLLKQAGDVEENPGPGSGEGRGSLLTCGDVEENPGPIDGGSGGSATMVSKGEELFTGVVPILVELDGDVNGHKFSVSGEGEGDATYGKLTLKLICTTGKLPVPWPTLVTTLGYGLQCFARYPDHMKQHDFFKSAMPEGYVQERTIFFKDDGNYKTRAEVKFDGDTLVNRIELKGIDFKEDGNILGHKLEYNYNSHNVYITADKQKNGIKANFKIRHNIEDGGVQLADHYQQNTPIGDGPVLLPDNHYLSYQSKLSKDPNEKRDHMVLLEFVTAAGITLGMDELYKGSGSGS

SEQ ID NO: 11 - protein, 343 aa, synthetic construct
  SOURCE 1..343
MEAKTYIGKLKSRKIVSNEDTYDIQTSTHNFFANDILVHNSEIGSGSGATNFSLLKQAGDVEENPGPGSGEGRGSLLTCGDVEENPGPIDGGSGGSATMVSKGEELFTGVVPILVELDGDVNGHKFSVSGEGEGDATYGKLTLKLICTTGKLPVPWPTLVTTLGYGLQCFARYPDHMKQHDFFKSAMPEGYVQERTIFFKDDGNYKTRAEVKFDGDTLVNRIELKGIDFKEDGNILGHKLEYNYNSHNVYITADKQKNGIKANFKIRHNIEDGGVQLADHYQQNTPIGDGPVLLPDNHYLSYQSKLSKDPNEKRDHMVLLEFVTAAGITLGMDELYKGSGSGS